European Patent Application EP 4 442 818 A1, published October 9, 2024. Title: TAQ POLYMERASE MUTANT, AND PREPARATION METHOD THEREFOR AND USE THEREOF. Applicant: DAAN GENE CO.,LTD. Application 22899855.5. The sequence listing filed with the application follows.

SEQUENCE LISTING (2 sequences)

SEQ ID NO: 1 - DNA, 2499 bp, Thermus aquaticus
atgcgtggcatgctgcctctgtttgaaccgaaaggccgcgtgttactggttgatggccatcatctggcctatcgtacctttcacgcactgaagggtctgaccacaagccgtggcgagccggttcaggccgtgtacggcttcgccaaaagcctgctgaaagccctgaaagaagacggcgatgccgtgatcgtggttttcgacgccaaggcaccgagctttcgtcatgaggcttatggtggctataaagccggtcgcgcaccgacaccggaggatttcccgcgccagctggccttaattaaagagctggtggatctgttaggcctggcccgcctggaggttccgggttatgaagccgacgacgtgctggccagcttagccaagaaggcagagaaagagggctatgaggtgcgcattctgaccgcagacaaggacctgtatcagctgctgagcgatcgcattcatgtgctgcatccggagggctacctgattaccccggcctggctgtgggaaaaatatggtctgcgcccggatcaatgggcagattatcgcgcactgacaggcgatgaaagcgataacctgccgggtgttaaaggcattggcgagaagacagcacgtaagctgctggaagaatggggtagcctggaagccctgttaaagaacctggaccgtctgaagccggcaatccgcgagaagattctggcccacatggatgatctgaagctgagttgggatctggccaaagttcgcacagacttaccgctggaagtggactttgccaagcgtcgtgaaccggaccgcgaacgtctgcgtgccttcttagaacgcctggaattcggtagcctgctgcacgaatttggtctgctggaaagcccgaaagccttagaagaagctccgtggccgcctccggaaggtgcctttgttggctttgttctgagccgcaaagagccgatgtgggcagatttactggccctggccgcagcacgcggtggtcgtgttcatcgtgccccggaaccgtataaagccctgcgcgacctgaaagaggcacgtggtctgttagcaaaggacctgagcgtgttagcactgcgtgaaggtctgggcttaccgcctggtgatgatccgatgctgctggcctacctgctggacccgagcaacaccacccctgagggtgtggcacgccgttatggtggtgaatggaccgaggaagcaggtgaacgcgccgcactgagtgagcgtctgtttgcaaacctgtggggccgtctggaaggcgaggaacgtctgctgtggctgtaccgcgaagtggaacgcccgctgagcgccgttttagcccacatggaggccaccggcgttcgcttagatgtggcctatctgcgcgccctgagcctggaagttgcagaagaaatcgcccgtctggaggcagaggtgtttcgtttagccggccatccgttcaacctgaatagccgcgaccagctggaacgcgtgctgtttgatgaactgggcttaccggccattggcaagaccgagaagaccggtaaacgtagtaccagtgcagccgttctggaagcactgcgtgaagcccaccctattgtggaaaagattctgcaatatcgcgagttaaccaaactgaagagcacctacatcgatcctctgcctgatctgattcacccgcgcaccggtcgtctgcacacccgctttaatcaaacagccacagccaccggtcgtctgagcagcagcgatccgaacttacagaacattccggtgcgcacccctctgggccaacgcattcgtcgcgccttcattgccgaagaaggctggttactggtggccctggactacagccagattgagctgcgtgttttagcccatctgagcggcgacgaaaacctgattcgcgtgtttcaagagggccgcgatattcatacagagaccgccagctggatgtttggtgttcctcgcgaagccgttgatccgctgatgcgccgcgcagccaaaacaattaacttcggtgtgctgtatggtatgagcgcccaccgtttaagccaggagctggccattccgtatgaagaggcccaggcatttatcgagcgctacttccagagtttccctaaggtgcgtgcatggatcgagaaaacactggaggaaggtcgccgtcgtggctacgtggaaaccctgtttggccgccgtcgctatgtgccggatctggaagcccgcgtgaaaagcgttcgtgaggcagcagagcgcatggcatttaatatgccggtgcagggtaccgcagccgacctgatgaaactggcaatggtgaagctgtttccgcgtctggaagagatgggcgcccgcatgttactgcaggtgcacgacgaactggttctggaggcaccgaaagaacgtgccgaagcagtggcacgcctggccaaagaggttatggaaggcgtttatccgttagccgttccgctggaggtggaggttggcattggcgaagactggctgagtgcaaaagaataa

SEQ ID NO: 2 - protein, 832 aa, Thermus aquaticus [sequence omitted]